European Patent Specification EP 4 271 651 B1, published October 23, 2024. Title: PRISTINE GRAPHENE BASED BIOSENSOR FOR BIOMARKER DETECTION AND RELATED CORE PARTICLES, MATERIALS COMPOSITIONS METHODS AND SYSTEMS. Applicant: KANSAS STATE UNIVERSITY RESEARCH FOUNDATION THE BOARD OF REGENTS OF THE UNIVERSITY OF TEXAS SYSTEM. The sequence listing filed with the application follows.

SEQUENCE LISTING (133 sequences)

SEQ ID NO: 1 - protein, 7 aa, Artificial Sequence
  Synthetic supramolecular recognition sequence
CQEQFWW

SEQ ID NO: 2 - protein, 13 aa, Artificial Sequence
  Synthetic supramolecular recognition sequence
PYFPRGSSYQGWN

SEQ ID NO: 3 - protein, 6 aa, Artificial Sequence
  Synthetic supramolecular recognition sequence
CCIQNQ

SEQ ID NO: 4 - protein, 8 aa, Artificial Sequence
  Synthetic supramolecular recognition sequence
AWYQPQFE

SEQ ID NO: 5 - protein, 6 aa, Artificial Sequence
  Synthetic supramolecular recognition sequence
EQQKRN

SEQ ID NO: 6 - protein, 8 aa, Artificial Sequence
  Synthetic supramolecular recognition sequence
CNHGKFYC

SEQ ID NO: 7 - protein, 8 aa, Artificial Sequence
  Synthetic supramolecular recognition sequence
NIYCNIAY

SEQ ID NO: 8 - protein, 8 aa, Artificial Sequence
  Synthetic supramolecular recognition sequence
KAYRWEFI

SEQ ID NO: 9 - protein, 9 aa, Artificial Sequence
  Synthetic supramolecular recognition sequence
IQNSGAPCH

SEQ ID NO: 10 - protein, 10 aa, Artificial Sequence
  Synthetic supramolecular recognition sequence
WQEAKNANQM

SEQ ID NO: 11 - protein, 8 aa, Artificial Sequence
  Synthetic supramolecular recognition sequence
RHQKTYSF

SEQ ID NO: 12 - protein, 10 aa, Artificial Sequence
  Synthetic supramolecular recognition sequence
  misc_feature (1)..(1): Xaa can be any naturally occurring amino acid
XLPPHWAGAL

SEQ ID NO: 13 - protein, 10 aa, Artificial Sequence
  Synthetic supramolecular recognition sequence
  misc_feature (1)..(1): Xaa can be any naturally occurring amino acid
XLPPHWAFAL

SEQ ID NO: 14 - protein, 28 aa, Artificial Sequence
  Synthetic supramolecular recognition sequence
LTELEKALNSIIDVYHKYSLIKGNFHAV

SEQ ID NO: 15 - protein, 30 aa, Artificial Sequence
  Synthetic supramolecular recognition sequence
GESMNFSDVFDSSEDYFVSVNTSYYSVDSE

SEQ ID NO: 16 - protein, 12 aa, Artificial Sequence
  Synthetic supramolecular recognition sequence
GTQWWVVCQQFG

SEQ ID NO: 17 - protein, 10 aa, Artificial Sequence
  Synthetic supramolecular recognition sequence
PGHWSDWSPS

SEQ ID NO: 18 - protein, 28 aa, Artificial Sequence
  Synthetic supramolecular recognition sequence
YFPEPVTVSGAGTFPAVLGSGQPPGKGL

SEQ ID NO: 19 - protein, 25 aa, Artificial Sequence
  Synthetic supramolecular recognition sequence
TAVYYCANRAGWGMGDYWGQGTQVT

SEQ ID NO: 20 - protein, 16 aa, Artificial Sequence
  Synthetic supramolecular recognition sequence
TASNYGAGYSTNDRHS

SEQ ID NO: 21 - protein, 10 aa, Artificial Sequence
  Synthetic supramolecular recognition sequence
NRPAQAWMLG

SEQ ID NO: 22 - protein, 20 aa, Artificial Sequence
  Synthetic supramolecular recognition sequence
AVYYCQQNNEDPRTFGGGTK

SEQ ID NO: 23 - protein, 13 aa, Artificial Sequence
  Synthetic supramolecular recognition sequence
AGDGYYPYAMDNW

SEQ ID NO: 24 - protein, 13 aa, Artificial Sequence
  Synthetic supramolecular recognition sequence
GWLPFGFILISAG

SEQ ID NO: 25 - protein, 11 aa, Artificial Sequence
  Synthetic supramolecular recognition sequence
YQQKPGQPPKL

SEQ ID NO: 26 - protein, 29 aa, Artificial Sequence
  Synthetic supramolecular recognition sequence
SVNWIRQPPGKALEWLAMIWGDGKIVYNS

SEQ ID NO: 27 - protein, 10 aa, Artificial Sequence
  Synthetic supramolecular recognition sequence
WLPFGFILIS

SEQ ID NO: 28 - protein, 14 aa, Artificial Sequence
  Synthetic supramolecular recognition sequence
TYYCQQWSGYPYTF

SEQ ID NO: 29 - protein, 13 aa, Artificial Sequence
  Synthetic supramolecular recognition sequence
SHFPYSQYQFWKN

SEQ ID NO: 30 - protein, 35 aa, Artificial Sequence
  Synthetic supramolecular recognition sequence
DMSDTNWWKGTSKGRTGLIPSNYVAEQAESIDNPL

SEQ ID NO: 31 - protein, 17 aa, Artificial Sequence
  Synthetic supramolecular recognition sequence
IAGKLQSAGSALWTDQL

SEQ ID NO: 32 - protein, 19 aa, Artificial Sequence
  Synthetic supramolecular recognition sequence
SSPKHVRFSWHQDAVTVTC

SEQ ID NO: 33 - protein, 10 aa, Artificial Sequence
  Synthetic supramolecular recognition sequence
AKCCPCQQWW

SEQ ID NO: 34 - protein, 15 aa, Artificial Sequence
  Synthetic supramolecular recognition sequence
VQEFYKDTYNKLKTK

SEQ ID NO: 35 - protein, 16 aa, Artificial Sequence
  Synthetic supramolecular recognition sequence
LNNHTASILNRMQANF

SEQ ID NO: 36 - protein, 19 aa, Artificial Sequence
  Synthetic supramolecular recognition sequence
VGIYILIAVGAVMMFVGFK

SEQ ID NO: 37 - protein, 18 aa, Artificial Sequence
  Synthetic supramolecular recognition sequence
NERNINITKDLLDLLVAH

SEQ ID NO: 38 - protein, 16 aa, Artificial Sequence
  Synthetic supramolecular recognition sequence
DINWVKQRPGQGLEWI

SEQ ID NO: 39 - protein, 16 aa, Artificial Sequence
  Synthetic supramolecular recognition sequence
VLLQGKNPDITKAWKL

SEQ ID NO: 40 - protein, 16 aa, Artificial Sequence
  Synthetic supramolecular recognition sequence
NLSRSRWFDFPFTREE

SEQ ID NO: 41 - protein, 8 aa, Artificial Sequence
  Synthetic protease consensus sequence
LAQAVVSS

SEQ ID NO: 42 - protein, 8 aa, Artificial Sequence
  Synthetic protease consensus sequence
GSQHIRAE

SEQ ID NO: 43 - protein, 12 aa, Artificial Sequence
  Synthetic protease consensus sequence
SLLKSRMVPNFN

SEQ ID NO: 44 - protein, 8 aa, Artificial Sequence
  Synthetic protease consensus sequence
GDSGLGRA

SEQ ID NO: 45 - protein, 8 aa, Artificial Sequence
  Synthetic protease consensus sequence
EVALVALK

SEQ ID NO: 46 - protein, 8 aa, Artificial Sequence
  Synthetic protease consensus sequence
LGLEGANL

SEQ ID NO: 47 - protein, 8 aa, Artificial Sequence
  Synthetic protease consensus sequence
AALGSAPG

SEQ ID NO: 48 - protein, 12 aa, Artificial Sequence
  Synthetic protease consensus sequence
SLLIFRSWANFN

SEQ ID NO: 49 - protein, 8 aa, Artificial Sequence
  Synthetic protease consensus sequence
VEPNSLEE

SEQ ID NO: 50 - protein, 8 aa, Artificial Sequence
  Synthetic protease consensus sequence
GEPLSLLP

SEQ ID NO: 51 - protein, 8 aa, Artificial Sequence
  Synthetic protease consensus sequence
IPVSLRSG

SEQ ID NO: 52 - protein, 8 aa, Artificial Sequence
  Synthetic protease consensus sequence
RPFSMIMG

SEQ ID NO: 53 - protein, 8 aa, Artificial Sequence
  Synthetic protease consensus sequence
VPLSLTMG

SEQ ID NO: 54 - protein, 8 aa, Artificial Sequence
  Synthetic protease consensus sequence
GPSGLRGA

SEQ ID NO: 55 - protein, 8 aa, Artificial Sequence
  Synthetic protease consensus sequence
VPLSLYSG

SEQ ID NO: 56 - protein, 8 aa, Artificial Sequence
  Synthetic protease consensus sequence
GAANLVRG

SEQ ID NO: 57 - protein, 9 aa, Artificial Sequence
  Synthetic protease consensus sequence
GVPLSLTMG

SEQ ID NO: 58 - protein, 11 aa, Artificial Sequence
  Synthetic protease consensus sequence
PQGLAGQRGIV

SEQ ID NO: 59 - protein, 8 aa, Artificial Sequence
  Synthetic protease consensus sequence
GPAGLRLA

SEQ ID NO: 60 - protein, 11 aa, Artificial Sequence
  Synthetic enzyme consensus sequence
RDIYAAPFFRK

SEQ ID NO: 61 - protein, 14 aa, Artificial Sequence
  Synthetic enzyme consensus sequence
AMERRRTSAARRSY

SEQ ID NO: 62 - protein, 13 aa, Artificial Sequence
  Synthetic enzyme consensus sequence
KARAAVSPQKRKA

SEQ ID NO: 63 - protein, 16 aa, Artificial Sequence
  Synthetic enzyme consensus sequence
RARKRRLSAPPLASGD

SEQ ID NO: 64 - protein, 15 aa, Artificial Sequence
  Synthetic enzyme consensus sequence
AKAGPPLSPRPPHVH

SEQ ID NO: 65 - protein, 15 aa, Artificial Sequence
  Synthetic enzyme consensus sequence
DLFIPDNYLKMKPAP

SEQ ID NO: 66 - protein, 15 aa, Artificial Sequence
  Synthetic enzyme consensus sequence
AELDPEDSMDMDMAP

SEQ ID NO: 67 - protein, 15 aa, Artificial Sequence
  Synthetic enzyme consensus sequence
EDEAEELSDEDEELK

SEQ ID NO: 68 - protein, 15 aa, Artificial Sequence
  Synthetic enzyme consensus sequence
AAGPAPLSPVPPVVH

SEQ ID NO: 69 - protein, 16 aa, Artificial Sequence
  Synthetic enzyme consensus sequence
DASRPPPLSPLPSPRA

SEQ ID NO: 70 - protein, 9 aa, Artificial Sequence
  Synthetic arginase consensus sequence
GRRRRRRRG

SEQ ID NO: 71 - protein, 17 aa, Artificial Sequence
  Synthetic supramolecular recognition sequence
AISGSGGSTYYANSVLG

SEQ ID NO: 72 - protein, 20 aa, Artificial Sequence
  Synthetic supramolecular recognition sequence
TNLGILHSMVARAVGNNTQG

SEQ ID NO: 73 - protein, 17 aa, Artificial Sequence
  Synthetic supramolecular recognition sequence
GIITYALSGGEIKILAG

SEQ ID NO: 74 - protein, 8 aa, Artificial Sequence
  Synthetic protease consensus sequence
SAVLLEAT

SEQ ID NO: 75 - protein, 8 aa, Artificial Sequence
  Synthetic protease consensus sequence
SQNYPIVQ

SEQ ID NO: 76 - protein, 12 aa, Artificial Sequence
  Synthetic arginase consensus sequence
GRRRRRRRGSSS

SEQ ID NO: 77 - protein, 24 aa, Artificial Sequence
  Synthetic supramolecular recognition sequence
AVYYCQQNNEDPRTFGGGTKSSSG

SEQ ID NO: 78 - protein, 21 aa, Artificial Sequence
  Synthetic supramolecular recognition sequence
QFVKDLLLHLKKLFREGRFNG

SEQ ID NO: 79 - protein, 21 aa, Artificial Sequence
  Synthetic supramolecular recognition sequence
QFVKDSLLHLKKLFREGRFNG

SEQ ID NO: 80 - protein, 21 aa, Artificial Sequence
  Synthetic supramolecular recognition sequence
QFVKDSLLHLSKLFREGRFNG

SEQ ID NO: 81 - protein, 21 aa, Artificial Sequence
  Synthetic supramolecular recognition sequence
QFVKDSLLHLSKLFRESRFNG

SEQ ID NO: 82 - protein, 8 aa, Artificial Sequence
  Synthetic enzyme consensus sequence
NVLHSWAV

SEQ ID NO: 83 - protein, 8 aa, Artificial Sequence
  Synthetic enzyme consensus sequence
ALQARPGP

SEQ ID NO: 84 - protein, 12 aa, Artificial Sequence
  Synthetic enzyme consensus sequence
SGVVIATVIVIT

SEQ ID NO: 85 - protein, 8 aa, Artificial Sequence
  Synthetic enzyme consensus sequence
RSARGLKG

SEQ ID NO: 86 - protein, 8 aa, Artificial Sequence
  Synthetic enzyme consensus sequence
RQSRIVFG

SEQ ID NO: 87 - protein, 8 aa, Artificial Sequence
  Synthetic enzyme consensus sequence
GEPVSGLP

SEQ ID NO: 88 - protein, 8 aa, Artificial Sequence
  Synthetic enzyme consensus sequence
VPMSMRGG

SEQ ID NO: 89 - protein, 8 aa, Artificial Sequence
  Synthetic enzyme consensus sequence
EPYHLMAL

SEQ ID NO: 90 - protein, 8 aa, Artificial Sequence
  Synthetic enzyme consensus sequence
RPLSLQTG

SEQ ID NO: 91 - protein, 8 aa, Artificial Sequence
  Synthetic enzyme consensus sequence
GPKNLKAP

SEQ ID NO: 92 - protein, 8 aa, Artificial Sequence
  Synthetic enzyme consensus sequence
GPANLVAP

SEQ ID NO: 93 - protein, 8 aa, Artificial Sequence
  Synthetic enzyme consensus sequence
LPQGLRTE

SEQ ID NO: 94 - protein, 8 aa, Artificial Sequence
  Synthetic enzyme consensus sequence
LPQKSQHG

SEQ ID NO: 95 - protein, 8 aa, Artificial Sequence
  Synthetic enzyme consensus sequence
LYYVSLSP

SEQ ID NO: 96 - protein, 8 aa, Artificial Sequence
  Synthetic enzyme consensus sequence
SYYVSLSP

SEQ ID NO: 97 - protein, 7 aa, Artificial Sequence
  Synthetic enzyme consensus sequence
RRRRRRR

SEQ ID NO: 98 - protein, 8 aa, Artificial Sequence
  Synthetic enzyme consensus sequence
EAFRSTGA

SEQ ID NO: 99 - protein, 8 aa, Artificial Sequence
  Synthetic enzyme consensus sequence
GTSRSAGG

SEQ ID NO: 100 - protein, 8 aa, Artificial Sequence
  Synthetic enzyme consensus sequence
YRFRILGG

SEQ ID NO: 101 - protein, 8 aa, Artificial Sequence
  Synthetic enzyme consensus sequence
IESKINGG

SEQ ID NO: 102 - protein, 8 aa, Artificial Sequence
  Synthetic enzyme consensus sequence
VRSRIVKG

SEQ ID NO: 103 - protein, 8 aa, Artificial Sequence
  Synthetic enzyme consensus sequence
TQPRIVGG

SEQ ID NO: 104 - protein, 8 aa, Artificial Sequence
  Synthetic enzyme consensus sequence
ALGRKLVG

SEQ ID NO: 105 - protein, 8 aa, Artificial Sequence
  Synthetic enzyme consensus sequence
STPPTPSP

SEQ ID NO: 106 - protein, 8 aa, Artificial Sequence
  Synthetic enzyme consensus sequence
VKAASLGK

SEQ ID NO: 107 - protein, 10 aa, Artificial Sequence
  Synthetic enzyme consensus sequence
TCCATCATCC

SEQ ID NO: 108 - protein, 8 aa, Artificial Sequence
  synthetic polypeptide
GLAGLVGP

SEQ ID NO: 109 - protein, 4 aa, Artificial Sequence
  synthetic polypeptide
DAFK

SEQ ID NO: 110 - protein, 8 aa, Artificial Sequence
  synthetic polypeptide
TSEEIRGG

SEQ ID NO: 111 - protein, 12 aa, Artificial Sequence
  synthetic polypeptide
SLLIFRSWANFN

SEQ ID NO: 112 - protein, 10 aa, Artificial Sequence
  synthetic polypeptide
SGKPILFFRL

SEQ ID NO: 113 - protein, 11 aa, Artificial Sequence
  synthetic polypeptide
SGSPAFLAKNR

SEQ ID NO: 114 - protein, 10 aa, Artificial Sequence
  synthetic polypeptide
SGKPIIFFRL

SEQ ID NO: 115 - protein, 8 aa, Artificial Sequence
  synthetic polypeptide
GAFRMCAG

SEQ ID NO: 116 - protein, 8 aa, Artificial Sequence
  synthetic polypeptide
EFVRSPTP

SEQ ID NO: 117 - protein, 8 aa, Artificial Sequence
  synthetic polypeptide
QFVRSPSG

SEQ ID NO: 118 - protein, 8 aa, Artificial Sequence
  synthetic polypeptide
AKLKAENN

SEQ ID NO: 119 - protein, 8 aa, Artificial Sequence
  synthetic polypeptide
EGLGQAGN

SEQ ID NO: 120 - protein, 8 aa, Artificial Sequence
  synthetic polypeptide
GKKGAVGE

SEQ ID NO: 121 - protein, 8 aa, Artificial Sequence
  synthetic polypeptide
GFFFWALG

SEQ ID NO: 122 - protein, 8 aa, Artificial Sequence
  synthetic polypeptide
GPLGMLSQ

SEQ ID NO: 123 - protein, 13 aa, Artificial Sequence
  synthetic polypeptide
GAGVPMSMRGGAG

SEQ ID NO: 124 - protein, 8 aa, Artificial Sequence
  synthetic polypeptide
GPSGLQTG

SEQ ID NO: 125 - protein, 11 aa, Artificial Sequence
  synthetic polypeptide
PQGLAGQRGIV

SEQ ID NO: 126 - protein, 12 aa, Artificial Sequence
  synthetic polypeptide
GPQGLAGQRGIV

SEQ ID NO: 127 - protein, 8 aa, Artificial Sequence
  synthetic polypeptide
IPESLRAG

SEQ ID NO: 128 - protein, 8 aa, Artificial Sequence
  synthetic polypeptide
ESDASQTG

SEQ ID NO: 129 - protein, 6 aa, Artificial Sequence
  synthetic polypeptide
SGASAC

SEQ ID NO: 130 - protein, 5 aa, Artificial Sequence
  synthetic polypeptide
SGRSA

SEQ ID NO: 131 - protein, 23 aa, Artificial Sequence
  synthetic eptide
KGTSKGRTGLIPSNYVAEQAEAG

SEQ ID NO: 132 - protein, 13 aa, Artificial Sequence
  synthetic peptide
GAGVPLSLYSGAG

SEQ ID NO: 133 - protein, 12 aa, Artificial Sequence
  Synthetic peptide
GAGRRRRRRRAG